European Patent Application EP 4 796 561 A1, published August 26, 2026. Title: anti-synaptotagmin-2 antibody. Applicant: Jiksak Bioengineering, Inc. The sequence listing filed with the application follows.

SEQUENCE LISTING (20 sequences)

SEQ ID NO: 1 - protein, 118 aa, synthetic construct
EVQLQQSGAELVRPGASVKLSCTASGFNIKDDYVHWVKQRPEQGLEWIGWIDPENGDTEYASKFQGKATITADASSNAAYLQLSSLTSEDTAAYYCTTDYYNNPFAYWGQGTLVTVSA

SEQ ID NO: 2 - protein, 106 aa, synthetic construct
QIVLTQSPAIMSASPGEKVTITCSASSSVSYMHWFQQKPGTSPKLWIYSTSKLASGVPVRFSGSGSGTSYSLTISRMEAEDAATYYCQQRSSYPFTFGSGTKLEIK

SEQ ID NO: 3 - protein, 6 aa, synthetic construct
KDDYVH

SEQ ID NO: 4 - protein, 17 aa, synthetic construct
WIDPENGDTEYASKFQG

SEQ ID NO: 5 - protein, 9 aa, synthetic construct
DYYNNPFAY

SEQ ID NO: 6 - protein, 10 aa, synthetic construct
SASSSVSYMH

SEQ ID NO: 7 - protein, 7 aa, synthetic construct
STSKLAS

SEQ ID NO: 8 - protein, 9 aa, synthetic construct
QQRSSYPFT

SEQ ID NO: 9 - protein, 419 aa, Homo sapiens
MRNIFKRNQEPIVAPATTTATMPIGPVDNSTESGGAGESQEDMFAKLKEKLFNEINKIPLPPWALIAIAVVAGLLLLTCCFCICKKCCCKKKKNKKEKGKGMKNAMNMKDMKGGQDDDDAETGLTEGEGEGEEEKEPENLGKLQFSLDYDFQANQLTVGVLQAAELPALDMGGTSDPYVKVFLLPDKKKKYETKVHRKTLNPAFNETFTFKVPYQELGGKTLVMAIYDFDRFSKHDIIGEVKVPMNTVDLGQPIEEWRDLQGGEKEEPEKLGDICTSLRYVPTAGKLTVCILEAKNLKKMDVGGLSDPYVKIHLMQNGKRLKKKKTTVKKKTLNPYFNESFSFEIPFEQIQKVQVVVTVLDYDKLGKNEAIGKIFVGSNATGTELRHWSDMLANPRRPIAQWHSLKPEEEVDALLGKNK

SEQ ID NO: 10 - protein, 422 aa, Mus musculus
MRNIFKRNQEPNVAPATTTATMPLAPVAPADNSTESTGPGESQEDMFAKLKEKFFNEINKIPLPPWALIAMAVVAGLLLLTCCFCICKKCCCKKKKNKKEKGKGMKNAMNMKDMKGGQDDDDAETGLTEGEGEGEEEKEPENLGKLQFSLDYDFQANQLTVGVLQAAELPALDMGGTSDPYVKVFLLPDKKKKYETKVHRKTLNPAFNETFTFKVPYQELAGKTLVMAIYDFDRFSKHDIIGEVKVPMNTVDLGQPIEEWRDLQGGEKEEPEKLGDICTSLRYVPTAGKLTVCILEAKNLKKMDVGGLSDPYVKIHLMQNGKRLKKKKTTVKKKTLNPYFNESFSFEIPFEQIQKVQVVVTVLDYDKLGKNEAIGKIFVGSNATGTELRHWSDMLANPRRPIAQWHSLKPEEEVDALLGKNK

SEQ ID NO: 11 - protein, 62 aa, Homo sapiens
MRNIFKRNQEPIVAPATTTATMPIGPVDNSTESGGAGESQEDMFAKLKEKLFNEINKIPLPP

SEQ ID NO: 12 - protein, 60 aa, Mus musculus
MRNIFKRNQEPNVAPATTTATMPLAPVAPADNSTESTGPGESQEDMFAKLKEKFFNEINK

SEQ ID NO: 13 - protein, 25 aa, Mus musculus
MRNIFKRNQEPIVAPATTTATMPIG

SEQ ID NO: 14 - protein, 26 aa, synthetic construct
  SITE 26: note = an additional Cysteine residue for binding to the carrier protein
MRNIFKRNQEPIVAPATTTATMPIGC

SEQ ID NO: 15 - protein, 63 aa, synthetic construct
  SITE 63: note = an additional Lysine residue bound to biotin
MRNIFKRNQEPIVAPATTTATMPIGPVDNSTESGGAGESQEDMFAKLKEKLFNEINKIPLPPK

SEQ ID NO: 16 - protein, 66 aa, synthetic construct
  SITE 66: note = an additional Lysine residue bound to biotin
MRNIFKRNQEPNVAPATTTATMPLAPVAPADNSTESTGPGESQEDMFAKLKEKFFNEINKIPLPPK

SEQ ID NO: 17 - protein, 59 aa, synthetic construct
  SITE 59: note = an additional Lysine residue bound to biotin
MVSESHHEALAAPPVTTVATVLPSNATEPASPGEGKEDAFSKLKEKFMNELHKIPLPPK

SEQ ID NO: 18 - DNA, 8353 bp, synthetic construct
  misc_feature 1028..1090: note = Leader sequence
  misc_feature 1091..2347: note = human SYT2 sequence
  source 1..8353: mol_type = other DNA
aacaaaatattaacgcttacaatttccattcgccattcaggctgcgcaactgttgggaagggcgatcggtgcgggcctcttcgctattacgccagctggcgaaagggggatgtgctgcaaggcgattaagttgggtaacgccagggttttcccagtcacgacgttgtaaaacgacggccagtgccaagctgatctatacattgaatcaatattggcaattagccatattagtcattggttatatagcataaatcaatattggctattggccattgcatacgttgtatctatatcataatatgtacatttatattggctcatgtccaatatgaccgccatgttgacattgattattgactagttattaatagtaatcaattacggggtcattagttcatagcccatatatggagttccgcgttacataacttacggtaaatggcccgcctggctgaccgcccaacgacccccgcccattgacgtcaataatgacgtatgttcccatagtaacgccaatagggactttccattgacgtcaatgggtggagtatttacggtaaactgcccacttggcagtacatcaagtgtatcatatgccaagtccgccccctattgacgtcaatgacggtaaatggcccgcctggcattatgcccagtacatgaccttacgggactttcctacttggcagtacatctacgtattagtcatcgctattaccatggtgatgcggttttggcagtacaccaatgggcgtggatagcggtttgactcacggggatttccaagtctccaccccattgacgtcaatgggagtttgttttggcaccaaaatcaacgggactttccaaaatgtcgtaataaccccgccccgttgacgcaaatgggcggtaggcgtgtacggtgggaggtctatataagcagagctcgtttagtgaaccgtcagaattttgtaatacgactcactatagggcggccgggaattcgtcgactggatccggtaccgaggagatctgccgccgcgatcgcatggagacagacacactcctgctatgggtactgctgctctgggttccaggttccactggtgacatgaggaacattttcaagaggaaccaggagcctattgtggctcctgccaccaccaccgccacgatgcccattggacccgtggacaactccactgagagtgggggtgctggggagagccaggaggacatgtttgccaaactgaaggagaagttattcaatgagataaacaagattcccttaccaccctgggcactgatcgccattgctgtggttgctgggctcctgcttctcacctgctgcttctgcatctgcaagaaatgctgctgcaagaagaagaagaacaagaaggagaagggcaaaggcatgaagaatgccatgaacatgaaggacatgaaagggggtcaggatgacgacgacgcagagacaggcctgactgagggggaaggtgaaggggaggaggagaaagagccagagaacctgggcaaactgcagttttccctggactatgattttcaggctaatcagcttactgtgggcgttctgcaggctgctgaactgcctgccctggacatgggaggcacctcagacccttatgtcaaggtcttcctccttcctgacaagaagaagaaatatgagaccaaagtccatcggaagacactgaaccctgccttcaatgaaaccttcaccttcaaggtgccataccaggagcttgggggcaaaactctggtgatggccatctatgactttgaccgcttctccaaacatgacatcattggagaggtaaaggtgcctatgaacacagtggacctcggccagcccattgaggagtggagagacctgcaaggcggggaaaaggaggagccggagaagctgggcgacatctgcacctccctgcgctatgtgcccacggccgggaagctcactgtctgcatcctggaggctaagaacctcaagaagatggacgtgggcggcctttcagacccgtacgtgaagatccacctgatgcagaatggcaagaggctcaagaagaagaagacaaccgtgaagaagaagaccctgaacccatacttcaacgagtccttcagctttgagatccccttcgagcagattcagaaagtccaggtagtggtcaccgtgctggactatgacaagctgggcaagaacgaagccataggcaagatcttcgtgggcagcaatgccacgggcacagagctgcggcactggtccgacatgctggccaacccccggaggcccatcgcccagtggcactcgctcaagcctgaggaggaggtggatgcactcctgggcaagaacaagacgcgtacgcggccgctcgagcagaaactcatctcagaagaggatctggcagcaaatgatatcctggattacaaggatgacgacgataaggtttaaacgtagcggccgcaaattccgcccctctccctcccccccccctaacgttactggccgaagccgcttggaataaggccggtgtgcgtttgtctatatgttattttccaccatattgccgtcttttggcaatgtgagggcccggaaacctggccctgtcttcttgacgagcattcctaggggtctttcccctctcgccaaaggaatgcaaggtctgttgaatgtcgtgaaggaagcagttcctctggaagcttcttgaagacaaacaacgtctgtagcgaccctttgcaggcagcggaaccccccacctggcgacaggtgcctctgcggccaaaagccacgtgtataagatacacctgcaaaggcggcacaaccccagtgccacgttgtgagttggatagttgtggaaagagtcaaatggctctcctcaagcgtattcaacaaggggctgaaggatgcccagaaggtaccccattgtatgggatctgatctggggcctcggtgcacatgctttacatgtgtttagtcgaggttaaaaaaacgtctaggccccccgaaccacggggacgtggttttcctttgaaaaacacgatgataatatggccacaaccatggagagcgacgagagcggcctgcccgccatggagatcgagtgccgcatcaccggcaccctgaacggcgtggagttcgagctggtgggcggcggagagggcacccccgagcagggccgcatgaccaacaagatgaagagcaccaaaggcgccctgaccttcagcccctacctgctgagccacgtgatgggctacggcttctaccacttcggcacctaccccagcggctacgagaaccccttcctgcacgccatcaacaacggcggctacaccaacacccgcatcgagaagtacgaggacggcggcgtgctgcacgtgagcttcagctaccgctacgaggccggccgcgtgatcggcgacttcaaggtgatgggcaccggcttccccgaggacagcgtgatcttcaccgacaagatcatccgcagcaacgccaccgtggagcacctgcaccccatgggcgataacgatctggatggcagcttcacccgcaccttcagcctgcgcgacggcggctactacagctccgtggtggacagccacatgcacttcaagagcgccatccaccccagcatcctgcagaacgggggccccatgttcgccttccgccgcgtggaggaggatcacagcaacaccgagctgggcatcgtggagtaccagcacgccttcaagaccccggatgcagatgccggtgaagaataatagccgctcatagctgtttcctgaacagatcccgggtggcatccctgtgacccctccccagtgcctctcctggccctggaagttgccactccagtgcccaccagccttgtcctaataaaattaagttgcatcattttgtctgactaggtgtccttctataatattatggggtggaggggggtggtatggagcaaggggcaagttgggaagacaacctgtagggcctgcggggtctattgggaaccaagctggagtgcagtggcacaatcttggctcactgcaatctccgcctcctgggttcaagcgattctcctgcctcagcctcccgagttgttgggattccaggcatgcatgaccaggctcagctaatttttgtttttttggtagagacggggtttcaccatattggccaggctggtctccaactcctaatctcaggtgatctacccaccttggcctcccaaattgctgggattacaggcgtgaaccactgctcccttccctgtccttctgattttaaaataactataccagcaggaggacgtccagacacagcataggctacctggccatgcccaaccggtgggacatttgagttgcttgcttggcactgtcctctcatgcgttgggtccactcagtagatgcctgttgaattgggtacgcggccagcttggctgtggaatgtgtgtcagttagggtgtggaaagtccccaggctccccagcaggcagaagtatgcaaagcatgcatctcaattagtcagcaaccaggtgtggaaagtccccaggctccccagcaggcagaagtatgcaaagcatgcatctcaattagtcagcaaccatagtcccgcccctaactccgcccatcccgcccctaactccgcccagttccgcccattctccgccccatggctgactaattttttttatttatgcagaggccgaggccgcctcggcctctgagctattccagaagtagtgaggaggcttttttggaggcctaggcttttgcaaaaagctcccgggagcttgtatatccattttcggatctgatcaagagacacgtacgaccatgaccgagtacaagcccacggtgcgcctcgccacccgcgacgacgtccccagggccgtacgcaccctcgccgccgcgttcgccgactaccccgccacgcgccacaccgtcgatccggaccgccacatcgagcgggtcaccgagctgcaagaactcttcctcacgcgcgtcgggctcgacatcggcaaggtgtgggtcgcggacgacggcgccgcggtggcggtctggaccacgccggagagcgtcgaagcgggggcggtgttcgccgagatcggcccgcgcatggccgagttgagcggttcccggctggccgcgcagcaacagatggaaggcctcctggcgccgcaccggcccaaggagcccgcgtggttcctggccaccgtcggcgtctcgcccgaccaccagggcaagggtctgggcagcgccgtcgtgctccccggagtggaggcggccgagcgcgccggggtgcccgccttcctggagacctccgcgccccgcaacctccccttctacgagcggctcggcttcaccgtcaccgccgacgtcgaggtgcccgaaggaccgcgcacctggtgcatgacccgcaagcccggtgcctgactgcagtgggactctggggttcgaaatgaccgaccaagcgacgcccaacctgccatcacgagatttcgattccaccgccgccttctatgaaaggttgggcttcggaatcgttttccgggacgccggctggatgatcctccagcgcggggatctcatgctggagttcttcgcccaccccaacttgtttattgcagcttataatggttacaaataaagcaatagcatcacaaatttcacaaataaagcatttttttcactgcattctagttgtggtttgtccaaactcatcaatgtatcttatcatgtctgtataccgtcgacctctagctagagcttggcgtaatcatggtcatagctgtttcctgtgtgaaattgttatccgctcacaattccacacaacatacgagccggaagcataaagtgtaaagcctggggtgcctaatgagtgagctaactcacattaattgcgttgcgctcactgcccgctttccagtcgggaaacctgtcgtgccagctgcattaatgaatcggccaacgcgcggggagaggcggtttgcgtattgggcgctcttccgcttcctcgctcactgactcgctgcgctcggtcgttcggctgcggcgagcggtatcagctcactcaaaggcggtaatacggttatccacagaatcaggggataacgcaggaaagaacatgtgagcaaaaggccagcaaaaggccaggaaccgtaaaaaggccgcgttgctggcgtttttccataggctccgcccccctgacgagcatcacaaaaatcgacgctcaagtcagaggtggcgaaacccgacaggactataaagataccaggcgtttccccctggaagctccctcgtgcgctctcctgttccgaccctgccgcttaccggatacctgtccgcctttctcccttcgggaagcgtggcgctttctcatagctcacgctgtaggtatctcagttcggtgtaggtcgttcgctccaagctgggctgtgtgcacgaaccccccgttcagcccgaccgctgcgccttatccggtaactatcgtcttgagtccaacccggtaagacacgacttatcgccactggcagcagccactggtaacaggattagcagagcgaggtatgtaggcggtgctacagagttcttgaagtggtggcctaactacggctacactagaagaacagtatttggtatctgcgctctgctgaagccagttaccttcggaaaaagagttggtagctcttgatccggcaaacaaaccaccgctggtagcggtggtttttttgtttgcaagcagcagattacgcgcagaaaaaaaggatctcaagaagatcctttgatcttttctacggggtctgacgctcagtggaacgaaaactcacgttaagggattttggtcatgagattatcaaaaaggatcttcacctagatccttttaaattaaaaatgaagttttaaatcaatctaaagtatatatgagtaaacttggtctgacagttaccaatgcttaatcagtgaggcacctatctcagcgatctgtctatttcgttcatccatagttgcctgactccccgtcgtgtagataactacgatacgggagggcttaccatctggccccagtgctgcaatgataccgcgagacccacgctcaccggctccagatttatcagcaataaaccagccagccggaagggccgagcgcagaagtggtcctgcaactttatccgcctccatccagtctattaattgttgccgggaagctagagtaagtagttcgccagttaatagtttgcgcaacgttgttgccattgctacaggcatcgtggtgtcacgctcgtcgtttggtatggcttcattcagctccggttcccaacgatcaaggcgagttacatgatcccccatgttgtgcaaaaaagcggttagctccttcggtcctccgatcgttgtcagaagtaagttggccgcagtgttatcactcatggttatggcagcactgcataattctcttactgtcatgccatccgtaagatgcttttctgtgactggtgagtactcaaccaagtcattctgagaatagtgtatgcggcgaccgagttgctcttgcccggcgtcaatacgggataataccgcgccacatagcagaactttaaaagtgctcatcattggaaaacgttcttcggggcgaaaactctcaaggatcttaccgctgttgagatccagttcgatgtaacccactcgtgcacccaactgatcttcagcatcttttactttcaccagcgtttctgggtgagcaaaaacaggaaggcaaaatgccgcaaaaaagggaataagggcgacacggaaatgttgaatactcatactcttcctttttcaatattattgaagcatttatcagggttattgtctcatgagcggatacatatttgaatgtatttagaaaaataaacaaataggggttccgcgcacatttccccgaaaagtgccacctgacgcgccctgtagcggcgcattaagcgcggcgggtgtggtggttacgcgcagcgtgaccgctacacttgccagcgccctagcgcccgctcctttcgctttcttcccttcctttctcgccacgttcgccggctttccccgtcaagctctaaatcgggggctccctttagggttccgatttagtgctttacggcacctcgaccccaaaaaacttgattagggtgatggttcacgtagtgggccatcgccctgatagacggtttttcgccctttgacgttggagtccacgttctttaatagtggactcttgttccaaactggaacaacactcaaccctatctcggtctattcttttgatttataagggattttgccgatttcggcctattggttaaaaaatgagctgatttaacaaaaatttaacgcgaatttt

SEQ ID NO: 19 - DNA, 63 bp, synthetic construct
  misc_feature 1..63: note = Leader sequence
  source 1..63: mol_type = other DNA
atggagacagacacactcctgctatgggtactgctgctctgggttccaggttccactggtgac

SEQ ID NO: 20 - DNA, 1257 bp, synthetic construct
  misc_feature 1..1257: note = human SYT2 sequence
  source 1..1257: mol_type = other DNA
atgaggaacattttcaagaggaaccaggagcctattgtggctcctgccaccaccaccgccacgatgcccattggacccgtggacaactccactgagagtgggggtgctggggagagccaggaggacatgtttgccaaactgaaggagaagttattcaatgagataaacaagattcccttaccaccctgggcactgatcgccattgctgtggttgctgggctcctgcttctcacctgctgcttctgcatctgcaagaaatgctgctgcaagaagaagaagaacaagaaggagaagggcaaaggcatgaagaatgccatgaacatgaaggacatgaaagggggtcaggatgacgacgacgcagagacaggcctgactgagggggaaggtgaaggggaggaggagaaagagccagagaacctgggcaaactgcagttttccctggactatgattttcaggctaatcagcttactgtgggcgttctgcaggctgctgaactgcctgccctggacatgggaggcacctcagacccttatgtcaaggtcttcctccttcctgacaagaagaagaaatatgagaccaaagtccatcggaagacactgaaccctgccttcaatgaaaccttcaccttcaaggtgccataccaggagcttgggggcaaaactctggtgatggccatctatgactttgaccgcttctccaaacatgacatcattggagaggtaaaggtgcctatgaacacagtggacctcggccagcccattgaggagtggagagacctgcaaggcggggaaaaggaggagccggagaagctgggcgacatctgcacctccctgcgctatgtgcccacggccgggaagctcactgtctgcatcctggaggctaagaacctcaagaagatggacgtgggcggcctttcagacccgtacgtgaagatccacctgatgcagaatggcaagaggctcaagaagaagaagacaaccgtgaagaagaagaccctgaacccatacttcaacgagtccttcagctttgagatccccttcgagcagattcagaaagtccaggtagtggtcaccgtgctggactatgacaagctgggcaagaacgaagccataggcaagatcttcgtgggcagcaatgccacgggcacagagctgcggcactggtccgacatgctggccaacccccggaggcccatcgcccagtggcactcgctcaagcctgaggaggaggtggatgcactcctgggcaagaacaag